European Patent Application EP 4 265 715 A1, published October 25, 2023. Title: A nucleic acid molecule containing a gene encoding a fusion protein of an antibody and a physiologically active protein. Applicant: JCR Pharmaceuticals Co., Ltd. The sequence listing filed with the application follows.

SEQUENCE LISTING (50 sequences)

SEQ ID NO: 1 - protein, 5 aa, Artificial Sequence
  Amino acid sequence of an exemplified linker 1
GGGGS

SEQ ID NO: 2 - protein, 6 aa, Artificial Sequence
  Amino acid sequence of an exemplified linker 2
GGGGGS

SEQ ID NO: 3 - protein, 5 aa, Artificial Sequence
  Amino acid sequence of an exemplified linker 3
SGGGG

SEQ ID NO: 4 - DNA, 145 bp, adeno-associated virus 2
ttggccactccctctctgcgcgctcgctcgctcactgaggccgggcgaccaaaggtcgcccgacgcccgggctttgcccgggcggcctcagtgagcgagcgagcgcgcagagagggagtggccaactccatcactaggggttcct

SEQ ID NO: 5 - DNA, 145 bp, adeno-associated virus 2
aggaacccctagtgatggagttggccactccctctctgcgcgctcgctcgctcactgaggccgggcgaccaaaggtcgcccgacgcccgggctttgcccgggcggcctcagtgagcgagcgagcgcgcagagagggagtggccaa

SEQ ID NO: 6 - DNA, 141 bp, Artificial Sequence
  A preferable example of nucleic acid sequence of the first Inverted Terminal Repeat (first ITR) , synthetic sequence
cctgcaggcagctgcgcgctcgctcgctcactgaggccgcccgggcaaagcccgggcgtcgggcgacctttggtcgcccggcctcagtgagcgagcgagcgcgcagagagggagtggccaactccatcactaggggttcct

SEQ ID NO: 7 - DNA, 141 bp, Artificial Sequence
  A preferable example of nucleic acid sequence of the second Inverted Terminal Repeat (second ITR) , synthetic sequence
aggaacccctagtgatggagttggccactccctctctgcgcgctcgctcgctcactgaggccgggcgaccaaaggtcgcccgacgcccgggctttgcccgggcggcctcagtgagcgagcgagcgcgcagctgcctgcagg

SEQ ID NO: 8 - DNA, 559 bp, Artificial Sequence
  Nucleic acid sequence of mouse alpha fetoprotein enhancer/mouse albumin promoter, synthetic sequence
agatcattttgatggcagagttcagtttaccgggtcacattgtacctgggaagattcaaggatttatggaaaaagtcaacaacaggagtcagagcagccggaaaagcatggactctgtacttaggactgcgctttgagcaatggcacagcaagctataaccctgtttgcagtcagcacacaaactgtggttcaaagctccactttatctcttcttgtggaattcagatatcagatcagttttgctcaaatgggagacaaagagattaagctcttatgtaaaatttgctgttttacataactttaatgaatggacaaagtcttgtgcatgggggtgggggtggggttagaggggaacagctccagatggcaaacatacgcaagggatttagtcaaacaactttttggcaaagatggtatgattttgtaatggggtaggaaccaatgaaatgcgaggtaagtatggttaataatctacagttattggttaaagaagtatattagagcgagtctttctgcacacagatcaccttcctatcaaccccactagcctctggcaaa

SEQ ID NO: 9 - DNA, 225 bp, Artificial Sequence
  Nucleic acid sequence of chicken beta actin/MVM chimeric intron, synthetic sequence
ggagtcgctgcgttgccttcgccccgtgccccgctccgcgccgcctcgcgccgcccgccccggctctgactgaccgcgttactcccacaggtgagcgggcgggacggcccttctcctccgggctgtaattagcaagaggtaagggtttaagggatggttggttggtggggtattaatgtttaattacctggagcacctgcctgaaatcactttttttcaggttgg

SEQ ID NO: 10 - DNA, 593 bp, Encephalomyocarditis virus
cccccccccctctccctcccccccccctaacgttactggccgaagccgcttggaataaggccggtgtgcgtttgtctatatgttattttccaccatattgccgtcttttggcaatgtgagggcccggaaacctggccctgtcttcttgacgagcattcctaggggtctttcccctctcgccaaaggaatgcaaggtctgttgaatgtcgtgaaggaagcagttcctctggaagcttcttgaagacaaacaacgtctgtagcgaccctttgcaggcagcggaaccccccacctggcgacaggtgcctctgcggccaaaagccacgtgtataagatacacctgcaaaggcggcacaaccccagtgccacgttgtgagttggatagttgtggaaagagtcaaatggctctcctcaagcgtattcaacaaggggctgaaggatgcccagaaggtaccccattgtatgggatctgatctggggcctcggtgcacatgctttacatgtgtttagtcgaggttaaaaaaacgtctaggccccccgaaccacggggacgtggttttcctttgaaaaacacgatgataatatggccacaacc

SEQ ID NO: 11 - protein, 760 aa, Homo sapiens
MMDQARSAFSNLFGGEPLSYTRFSLARQVDGDNSHVEMKLAVDEEENADNNTKANVTKPKRCSGSICYGTIAVIVFFLIGFMIGYLGYCKGVEPKTECERLAGTESPVREEPGEDFPAARRLYWDDLKRKLSEKLDSTDFTGTIKLLNENSYVPREAGSQKDENLALYVENQFREFKLSKVWRDQHFVKIQVKDSAQNSVIIVDKNGRLVYLVENPGGYVAYSKAATVTGKLVHANFGTKKDFEDLYTPVNGSIVIVRAGKITFAEKVANAESLNAIGVLIYMDQTKFPIVNAELSFFGHAHLGTGDPYTPGFPSFNHTQFPPSRSSGLPNIPVQTISRAAAEKLFGNMEGDCPSDWKTDSTCRMVTSESKNVKLTVSNVLKEIKILNIFGVIKGFVEPDHYVVVGAQRDAWGPGAAKSGVGTALLLKLAQMFSDMVLKDGFQPSRSIIFASWSAGDFGSVGATEWLEGYLSSLHLKAFTYINLDKAVLGTSNFKVSASPLLYTLIEKTMQNVKHPVTGQFLYQDSNWASKVEKLTLDNAAFPFLAYSGIPAVSFCFCEDTDYPYLGTTMDTYKELIERIPELNKVARAAAEVAGQFVIKLTHDVELNLDYERYNSQLLSFVRDLNQYRADIKEMGLSLQWLYSARGDFFRATSRLTTDFGNAEKTDRFVMKKLNDRVMRVEYHFLSPYVSPKESPFRHVFWGSGSHTLPALLENLKLRKQNNGAFNETLFRNQLALATWTIQGAANALSGDVWDIDNEF

SEQ ID NO: 12 - protein, 226 aa, Artificial Sequence
  An example of amino acid sequence of Fab region of the heavy chain of anti-hTfR antibody
EVQLVQSGAEVKKPGESLKISCKGSGYSFMNYWLGWVRQMPGKGLEWMGDIYPGGDYPTYSEKFKVQVTISADKSISTAYLQLSSLKASDTAMYYCARSGNYDEVAYWGQGTLVTVSSASTKGPSVFPLAPSSKSTSGGTAALGCLVKDYFPEPVTVSWNSGALTSGVHTFPAVLQSSGLYSLSSVVTVPSSSLGTQTYICNVNHKPSNTKVDKKVEPKSCDKTHT

SEQ ID NO: 13 - protein, 15 aa, Artificial Sequence
  Amino acid sequence of an exemplified linker 4
GGGGSGGGGSGGGGS

SEQ ID NO: 14 - protein, 525 aa, Homo sapiens
SETQANSTTDALNVLLIIVDDLRPSLGCYGDKLVRSPNIDQLASHSLLFQNAFAQQAVCAPSRVSFLTGRRPDTTRLYDFNSYWRVHAGNFSTIPQYFKENGYVTMSVGKVFHPGISSNHTDDSPYSWSFPPYHPSSEKYENTKTCRGPDGELHANLLCPVDVLDVPEGTLPDKQSTEQAIQLLEKMKTSASPFFLAVGYHKPHIPFRYPKEFQKLYPLENITLAPDPEVPDGLPPVAYNPWMDIRQREDVQALNISVPYGPIPVDFQRKIRQSYFASVSYLDTQVGRLLSALDDLQLANSTIIAFTSDHGWALGEHGEWAKYSNFDVATHVPLIFYVPGRTASLPEAGEKLFPYLDPFDSASQLMEPGRQSMDLVELVSLFPTLAGLAGLQVPPRCPVPSFHVELCREGKNLLKHFRFRDLEEDPYLPGNPRELIAYSQYPRPSDIPQWNSDKPSLKDIKIMGYSIRTIDYRYTVWVGFNPDEFLANFSDIHAGELYFVDSDPLQDHNMYNDSQGGDLFQLLMP

SEQ ID NO: 15 - protein, 219 aa, Artificial Sequence
  An example of amino acid sequence of the light chain of anti-hTfR antibody
DIVMTQTPLSLSVTPGQPASISCRSSQSLVHSNGNTYLHWYLQKPGQSPQLLIYKVSNRFSGVPDRFSGSGSGTDFTLKISRVEAEDVGVYYCSQSTHVPWTFGQGTKVEIKRTVAAPSVFIFPPSDEQLKSGTASVVCLLNNFYPREAKVQWKVDNALQSGNSQESVTEQDSKDSTYSLSSTLTLSKADYEKHKVYACEVTHQGLSSPVTKSFNRGEC

SEQ ID NO: 16 - protein, 226 aa, Artificial Sequence; identical to SEQ ID NO: 12
  An example of amino acid sequence of the heavy chain of anti-hTfR antibody

SEQ ID NO: 17 - DNA, 208 bp, Bos taurus
ctgtgccttctagttgccagccatctgttgtttgcccctcccccgtgccttccttgaccctggaaggtgccactcccactgtcctttcctaataaaatgaggaaattgcatcgcattgtctgagtaggtgtcattctattctggggggtggggtggggcaggacagcaagggggaggattgggaagacaatagcaggcatgctgggga

SEQ ID NO: 18 - DNA, 4744 bp, Artificial Sequence
  Nucleic acid sequence of the DNA fragment synthesized for construction of pAAV-mMAP-Fab-hI2S vector, synthetic sequence
atcgatatcaagcttagatcattttgatggcagagttcagtttaccgggtcacattgtacctgggaagattcaaggatttatggaaaaagtcaacaacaggagtcagagcagccggaaaagcatggactctgtacttaggactgcgctttgagcaatggcacagcaagctataaccctgtttgcagtcagcacacaaactgtggttcaaagctccactttatctcttcttgtggaattcagatatcagatcagttttgctcaaatgggagacaaagagattaagctcttatgtaaaatttgctgttttacataactttaatgaatggacaaagtcttgtgcatgggggtgggggtggggttagaggggaacagctccagatggcaaacatacgcaagggatttagtcaaacaactttttggcaaagatggtatgattttgtaatggggtaggaaccaatgaaatgcgaggtaagtatggttaataatctacagttattggttaaagaagtatattagagcgagtctttctgcacacagatcaccttcctatcaaccccactagcctctggcaaaggtaccagtgtacagggagtcgctgcgttgccttcgccccgtgccccgctccgcgccgcctcgcgccgcccgccccggctctgactgaccgcgttactcccacaggtgagcgggcgggacggcccttctcctccgggctgtaattagcaagaggtaagggtttaagggatggttggttggtggggtattaatgtttaattacctggagcacctgcctgaaatcactttttttcaggttggacgcgtcgccaccatgggttggagcctcatcttgctcttccttgtcgctgttgctacgcgagtcggcagcgaggtgcaactagtgcagtctggagcagaggtgaaaaagcccggggagtctctgaagatttcctgtaagggttctggatacagctttatgaactactggctgggatgggtgcgccagatgcccgggaaaggcctggagtggatgggggacatctaccccggcggagactaccctacatacagcgagaagttcaaggtccaggtcaccatctcagccgacaagtccatcagcaccgcctacctgcagttgagcagcctgaaggcctcggacaccgccatgtattactgtgcgagatcaggcaattacgacgaagtggcctactggggccaaggaaccctggtcaccgtctcctcagctagcaccaagggcccatcggtcttccccctggcaccctcctccaagagcacctctgggggcacagcggccctgggctgcctggtcaaggactacttccccgaaccggtgacggtgtcgtggaactcaggcgccctgaccagcggcgtgcacaccttcccggctgtcctacagtcctcaggactctactccctcagcagcgtggtgaccgtgccctccagcagcttgggcacccagacctacatctgcaacgtgaatcacaagcccagcaacaccaaggtggacaagaaagttgagccgaagagctgtgataagacgcatacgggtggcggagggtctggaggtggcggatcaggcggaggtggatcttccgaaacgcaggccaactcgaccacagatgctctgaacgttcttctcatcatcgtggatgacctgcgcccctccctgggctgttatggggataagctggtgaggtccccaaatattgaccaactggcatcccacagcctcctcttccagaatgcctttgcgcagcaagcagtgtgcgccccgagccgcgtttctttcctcactggcaggagacctgacaccacccgcctgtacgacttcaactcctactggagggtgcacgctggaaacttctccaccatcccccagtacttcaaggagaatggctatgtgaccatgtcggtgggaaaagtctttcaccctgggatatcttctaaccataccgatgattctccgtatagctggtcttttccaccttatcatccttcctctgagaagtatgaaaacactaagacatgtcgagggccagatggagaactccatgccaacctgctttgccctgtggatgtgctggatgttcccgagggcaccttgcctgacaaacagagcactgagcaagccatacagttgttggaaaagatgaaaacgtcagccagtcctttcttcctggccgttgggtatcataagccacacatccccttcagataccccaaggaatttcagaagttgtatcccttggagaacatcaccctggcccccgatcccgaggtccctgatggcctaccccctgtggcctacaacccctggatggacatcaggcaacgggaagacgtccaagccttaaacatcagtgtgccgtatggtccaattcctgtggactttcagcggaaaatccgccagagctactttgcctctgtgtcatatttggatacacaggtcggccgcctcttgagtgctttggacgatcttcagctggccaacagcaccatcattgcatttacctcggatcatgggtgggctctaggtgaacatggagaatgggccaaatacagcaattttgatgttgctacccatgttcccctgatattctatgttcctggaaggacggcttcacttccggaggcaggcgagaagcttttcccttacctcgacccttttgattccgcctcacagttgatggagccaggcaggcaatccatggaccttgtggaacttgtgtctctttttcccacgctggctggacttgcaggactgcaggttccacctcgctgccccgttccttcatttcacgttgagctgtgcagagaaggcaagaaccttctgaagcattttcgattccgtgacttggaagaagatccgtacctccctggtaatccccgtgaactgattgcctatagccagtatccccggccttcagacatccctcagtggaattctgacaagccgagtttaaaagatataaagatcatgggctattccatacgcaccatagactataggtatactgtgtgggttggcttcaatcctgatgaatttctagctaacttttctgacatccatgcaggggaactgtattttgtggattctgacccattgcaggatcacaatatgtataatgattcccaaggtggagaccttttccagttgttgatgccttaataagcggccgccccccccccctctccctcccccccccctaacgttactggccgaagccgcttggaataaggccggtgtgcgtttgtctatatgttattttccaccatattgccgtcttttggcaatgtgagggcccggaaacctggccctgtcttcttgacgagcattcctaggggtctttcccctctcgccaaaggaatgcaaggtctgttgaatgtcgtgaaggaagcagttcctctggaagcttcttgaagacaaacaacgtctgtagcgaccctttgcaggcagcggaaccccccacctggcgacaggtgcctctgcggccaaaagccacgtgtataagatacacctgcaaaggcggcacaaccccagtgccacgttgtgagttggatagttgtggaaagagtcaaatggctctcctcaagcgtattcaacaaggggctgaaggatgcccagaaggtaccccattgtatgggatctgatctggggcctcggtgcacatgctttacatgtgtttagtcgaggttaaaaaaacgtctaggccccccgaaccacggggacgtggttttcctttgaaaaacacgatgataatatggccacaaccatgggctggagctggattctgctgttcctcctgagcgtgacagcaggagtgcacagcgacatcgtgatgacccagactcccctgagcctgagcgtgacacctggccagcctgccagcatcagctgcagaagctctcagagcctggtgcacagcaacggcaacacctacctgcactggtatctgcagaagcccggccagagccctcagctgctgatctacaaggtgtccaacagattcagcggcgtgcccgacagattctccggcagcggctctggcaccgacttcaccctgaagatttccagagtggaagccgaggacgtgggcgtgtactactgcagccagagcacccacgtgccctggacattcggccagggcaccaaggtggaaatcaagagaaccgtggccgctcccagcgtgttcatcttcccacctagcgacgagcagctgaagtccggcacagcctctgtcgtgtgcctgctgaacaacttctacccccgcgaggccaaggtgcagtggaaggtggacaacgccctgcagagcggcaacagccaggaaagcgtgaccgagcaggactccaaggacagcacctacagcctgagcagcaccctgaccctgagcaaggccgactacgagaagcacaaggtgtacgcctgcgaagtgacccaccagggcctgtctagccccgtgaccaagagcttcaacagaggcgagtgctaaatttaaatgcggccgcatttaaatctgtgccttctagttgccagccatctgttgtttgcccctcccccgtgccttccttgaccctggaaggtgccactcccactgtcctttcctaataaaatgaggaaattgcatcgcattgtctgagtaggtgtcattctattctggggggtggggtggggcaggacagcaagggggaggattgggaagacaatagcaggcatgctggggaagatct

SEQ ID NO: 19 - DNA, 2820 bp, Artificial Sequence
  Nucleic acid sequence of the DNA fragment synthesized for construction of pR2(mod)C6 vector, synthetic sequence
agcgctcggaccgggcgcgctcactggccgtcgttttacaacgtcgtgactgggaaaaccctgtacaggctgaccggtgttgcctaggtgaatggcgaatggtcaggtggcacttttcggggaaatgtgcgcggaacccctatttgtttatttttctaaatacattcaaatatgtatccgctcatgagacaataaccctgataaatgcttcaataatattgaaaaaggaagagtatgagtattcaacatttccgtgtcgcccttattcccttttttgcggcattttgccttcctgtttttgctcacccagaaacgctggtgaaagtaaaagatgctgaagatcagttgggtgcacgagtgggttacatcgaactggatctcaacagcggtaagatccttgagagttttcgccccgaagaacgttttccaatgatgagcacttttaaagttctgctatgtggcgcggtattatcccgtattgacgccgggcaagagcaactcggtcgccgcatacactattctcagaatgacttggttgagtactcaccagtcacagaaaagcatcttacggatggcatgacagtaagagaattatgcagtgctgccataaccatgagtgataacactgcggccaacttacttctgacaacgatcggaggaccgaaggagctaaccgcttttttgcacaacatgggggatcatgtaactcgccttgatcgttgggaaccggagctgaatgaagccataccaaacgacgagcgtgacaccacgatgcctgtagcaatggcaacaacgttgcgcaaactattaactggcgaactacttactctagcttcccggcaacaattaatagactggatggaggcggataaagttgcaggaccacttctgcgctcggcccttccggctggctggtttattgctgataaatctggagccggtgagcgtgggtctcgcggtatcattgcagcactggggccagatggtaagccctcccgtatcgtagttatctacacgacggggagtcaggcaactatggatgaacgaaatagacagatcgctgagataggtgcctcactgattaagcattggtaactgtcagaccaagtttactcatatatactttagattgatttaaaacttcatttttaatttaaaaggatctaggtgaagatcctttttgataatctcatgaccaaaatcccttaacgtgagttttcgttccactgagcgtcagaccccgtagaaaagatcaaaggatcttcttgagatcctttttttctgcgcgtaatctgctgcttgcaaacaaaaaaaccaccgctaccagcggtggtttgtttgccggatcaagagctaccaactctttttccgaaggtaactggcttcagcagagcgcagataccaaatactgttcttctagtgtagccgtagttaggccaccacttcaagaactctgtagcaccgcctacatacctcgctctgctaatcctgttaccagtggctgctgccagtggcgataagtcgtgtcttaccgggttggactcaagacgatagttaccggataaggcgcagcggtcgggctgaacggggggttcgtgcacacagcccagcttggagcgaacgacctacaccgaactgagatacctacagcgtgagctatgagaaagcgccacgcttcccgaagggagaaaggcggacaggtatccggtaagcggcagggtcggaacaggagagcgcacgagggagcttccagggggaaacgcctggtatctttatagtcctgtcgggtttcgccacctctgacttgagcgtcgatttttgtgatgctcgtcaggggggcggagcctatggaaaaacgccagcaacgcggcctttttacggttcctggccttttgctggccttttgctcacatgttctttcctgcgttatcccctgattctgtggataaccgtattaccgcctttgagtgagctgataccgctcgccgcagccgaacgaccgagcgcagcgagtcagtgagcgaggaagcggaagagcgcccaatacgcaaaccgcctctccccgcgcgttggccgattcattaatgcagctggcacgacaggtttcccgactggaaagcgggcagtgagcgcaacgcaattaatgtgagttagctcactcattaggcaccccaggctttacactttatgcttccggctcgtatgttgtgtggaattgtgagcggataacaatttcacacaggaaacagctatgaccatgattacgccaacggaccgggaggggtggagtcgtgacgtgaattacgtcatagggttagggaggtcctgtattagaggtcacgtgagtgttttgcgacattttgcgacaccatgtggtctcgctgggggggggggcccgagtgagcacgcagggtctccattttgaagcgggaggtttgaacgcgcagccgccacgccggggttttacgagattgtgattaaggtccccagcgaccttgacgagcatctgcccggcatttctgacagctttgtgaactgggtggccgagaaggaatgggagttgccgccagattctgacatggatctgaatctgattgagcaggcacccctgaccgtggccgagaagctgcagcgcgactttctgacggaatggcgccgtgtgagtaaggccccggaggcccttttctttgtgcaatttgagaagggagagagctacttccacatgcacgtgctcgtggaaaccaccggggtgaaatccatggttttgggacgtttcctgagtcagattcgcgaaaaactgattcagagaatttaccgcgg

SEQ ID NO: 20 - DNA, 2911 bp, Artificial Sequence
  Nucleic acid sequence of the DNA fragment synthesized for construction of pR2(mod)C8 vector, synthetic sequence
aagcttcgatcaactacgcagacaggtaccaaaacaaatgttctcgtcacgtgggcatgaatctgatgctgtttccctgcagacaatgcgagagaatgaatcagaattcaaatatctgcttcactcacggacagaaagactgtttagagtgctttcccgtgtcagaatctcaacccgtttctgtcgtcaaaaaggcgtatcagaaactgtgctacattcatcatatcatgggaaaggtgccagacgcttgcactgcctgcgatctggtcaatgtggatttggatgactgcatctttgaacaataaatgatttaaatcaggtatggctgccgatggttatcttccagattggctcgaggacaacctctctgagggcattcgcgagtggtgggacttgaaacctggagccccgaaacccaaagccaaccagcaaaagcaggacgacggccggggtctggtgcttcctggctacaagtacctcggacccttcaacggactcgacaagggggagcccgtcaacgcggcggatgcagcggccctcgagcacgacaaggcctacgaccagcagctcaaagcgggtgacaatccgtacctgcggtataaccacgccgacgccgagtttcaggagcgtctgcaagaagatacgtcttttgggggcaacctcgggcgagcagtcttccaggccaagaagagggttctcgaaccttttggtctggttgaggaaggtgctaagacggctcctggaaagaaacgtccggtagagcagtcgccacaagagccagactcctcctcgggcattggcaagacaggccagcagcccgctaaaaagagactcaattttggtcagactggcgactcagagtcagtccccgacccacaacctctcggagaacctccagcaacccccgctgctgtgggacctactacaatggcttcaggcggtggcgcaccaatggcagacaataacgaaggcgccgacggagtgggtaatgcctcaggaaattggcattgcgattccacatggctgggcgacagagtcatcaccaccagcacccgaacatgggccttgcccacctataacaaccacctctacaagcaaatctccagtgcttcaacgggggccagcaacgacaaccactacttcggctacagcaccccctgggggtattttgatttcaacagattccactgccatttctcaccacgtgactggcagcgactcatcaacaacaattggggattccggcccaagagactcaacttcaagctcttcaacatccaagtcaaggaggtcacgacgaatgatggcgtcacgaccatcgctaataaccttaccagcacggttcaagtcttctcggactcggagtaccagttgccgtacgtcctcggctctgcgcaccagggctgcctccctccgttcccggcggacgtgttcatgattccgcagtacggctacctaacgctcaacaatggcagccaggcagtgggacggtcatccttttactgcctggaatatttcccatcgcagatgctgagaacgggcaataactttaccttcagctacaccttcgaggacgtgcctttccacagcagctacgcgcacagccagagcctggaccggctgatgaatcctctcatcgaccagtacctgtattacctgaacagaactcagaatcagtccggaagtgcccaaaacaaggacttgctgtttagccgggggtctccagctggcatgtctgttcagcccaaaaactggctacctggaccctgttaccggcagcagcgcgtttctaaaacaaaaacagacaacaacaacagcaactttacctggactggtgcttcaaaatataaccttaatgggcgtgaatctataatcaaccctggcactgctatggcctcacacaaagacgacaaagacaagttctttcccatgagcggtgtcatgatttttggaaaggagagcgccggagcttcaaacactgcattggacaatgtcatgatcacagacgaagaggaaatcaaagccactaaccccgtggccaccgaaagatttgggactgtggcagtcaatctccagagcagcagcacagaccctgcgaccggagatgtgcatgttatgggagccttacctggaatggtgtggcaagacagagacgtatacctgcagggtcctatttgggccaaaattcctcacacggatggacactttcacccgtctcctctcatgggcggctttggacttaagcacccgcctcctcagatcctcatcaaaaacacgcctgttcctgcgaatcctccggcagagttttcggctacaaagtttgcttcattcatcacccagtattccacaggacaagtgagcgtggagattgaatgggagctgcagaaagaaaacagcaaacgctggaatcccgaagtgcagtatacatctaactatgcaaaatctgccaacgttgatttcactgtggacaacaatggactttatactgagcctcgccccattggcacccgttacctcacccgtcccctgtaattgcttgttaatcaataaaccgtttaattcgtttcagttgaactttggtctctgcgtatttctttcttatctagtttccatggctacgtagataagtagcatggcgggttaatcattaactacagcccgggcgtttaaacagcgggcggaggggtggagtcgtgacgtgaattacgtcatagggttagggaggtcctgtattagaggtcacgtgagtgttttgcgacattttgcgacaccatgtggtctcgctgggggggggggcccgagtgagcacgcagggtctccattttgaagcgggaggtttgaacgagcgctcggaccgggcgcgctcactggccgtcgttttacaacgtcgtgactgggaaaaccctgtaca

SEQ ID NO: 21 - DNA, 2038 bp, Artificial Sequence
  Nucleic acid sequence of Rep region of serotype 2 AAV containing p5 promoter, synthetic sequence
ggaggggtggagtcgtgacgtgaattacgtcatagggttagggaggtcctgtattagaggtcacgtgagtgttttgcgacattttgcgacaccatgtggtctcgctgggggggggggcccgagtgagcacgcagggtctccattttgaagcgggaggtttgaacgcgcagccgccacgccggggttttacgagattgtgattaaggtccccagcgaccttgacgagcatctgcccggcatttctgacagctttgtgaactgggtggccgagaaggaatgggagttgccgccagattctgacatggatctgaatctgattgagcaggcacccctgaccgtggccgagaagctgcagcgcgactttctgacggaatggcgccgtgtgagtaaggccccggaggcccttttctttgtgcaatttgagaagggagagagctacttccacatgcacgtgctcgtggaaaccaccggggtgaaatccatggttttgggacgtttcctgagtcagattcgcgaaaaactgattcagagaatttaccgcgggatcgagccgactttgccaaactggttcgcggtcacaaagaccagaaatggcgccggaggcgggaacaaggtggtggatgagtgctacatccccaattacttgctccccaaaacccagcctgagctccagtgggcgtggactaatatggaacagtatttaagcgcctgtttgaatctcacggagcgtaaacggttggtggcgcagcatctgacgcacgtgtcgcagacgcaggagcagaacaaagagaatcagaatcccaattctgatgcgccggtgatcagatcaaaaacttcagccaggtacatggagctggtcgggtggctcgtggacaaggggattacctcggagaagcagtggatccaggaggaccaggcctcatacatctccttcaatgcggcctccaactcgcggtcccaaatcaaggctgccttggacaatgcgggaaagattatgagcctgactaaaaccgcccccgactacctggtgggccagcagcccgtggaggacatttccagcaatcggatttataaaattttggaactaaacgggtacgatccccaatatgcggcttccgtctttctgggatgggccacgaaaaagttcggcaagaggaacaccatctggctgtttgggcctgcaactaccgggaagaccaacatcgcggaggccatagcccacactgtgcccttctacgggtgcgtaaactggaccaatgagaactttcccttcaacgactgtgtcgacaagatggtgatctggtgggaggaggggaagatgaccgccaaggtcgtggagtcggccaaagccattctcggaggaagcaaggtgcgcgtggaccagaaatgcaagtcctcggcccagatagacccgactcccgtgatcgtcacctccaacaccaacatgtgcgccgtgattgacgggaactcaacgaccttcgaacaccagcagccgttgcaagaccggatgttcaaatttgaactcacccgccgtctggatcatgactttgggaaggtcaccaagcaggaagtcaaagactttttccggtgggcaaaggatcacgtggttgaggtggagcatgaattctacgtcaaaaagggtggagccaagaaaagacccgcccccagtgacgcagatataagtgagcccaaacgggtgcgcgagtcagttgcgcagccatcgacgtcagacgcggaagcttcgatcaactacgcagacaggtaccaaaacaaatgttctcgtcacgtgggcatgaatctgatgctgtttccctgcagacaatgcgagagaatgaatcagaattcaaatatctgcttcactcacggacagaaagactgtttagagtgctttcccgtgtcagaatctcaacccgtttctgtcgtcaaaaaggcgtatcagaaactgtgctacattcatcatatcatgggaaaggtgccagacgcttgcactgcctgcgatctggtcaatgtggatttggatgactgcatctttgaacaa

SEQ ID NO: 22 - DNA, 2214 bp, adeno-associated virus 8
atggctgccgatggttatcttccagattggctcgaggacaacctctctgagggcattcgcgagtggtgggcgctgaaacctggagccccgaagcccaaagccaaccagcaaaagcaggacgacggccggggtctggtgcttcctggctacaagtacctcggacccttcaacggactcgacaagggggagcccgtcaacgcggcggacgcagcggccctcgagcacgacaaggcctacgaccagcagctgcaggcgggtgacaatccgtacctgcggtataaccacgccgacgccgagtttcaggagcgtctgcaagaagatacgtcttttgggggcaacctcgggcgagcagtcttccaggccaagaagcgggttctcgaacctctcggtctggttgaggaaggcgctaagacggctcctggaaagaagagaccggtagagccatcaccccagcgttctccagactcctctacgggcatcggcaagaaaggccaacagcccgccagaaaaagactcaattttggtcagactggcgactcagagtcagttccagaccctcaacctctcggagaacctccagcagcgccctctggtgtgggacctaatacaatggctgcaggcggtggcgcaccaatggcagacaataacgaaggcgccgacggagtgggtagttcctcgggaaattggcattgcgattccacatggctgggcgacagagtcatcaccaccagcacccgaacctgggccctgcccacctacaacaaccacctctacaagcaaatctccaacgggacatcgggaggagccaccaacgacaacacctacttcggctacagcaccccctgggggtattttgactttaacagattccactgccacttttcaccacgtgactggcagcgactcatcaacaacaactggggattccggcccaagagactcagcttcaagctcttcaacatccaggtcaaggaggtcacgcagaatgaaggcaccaagaccatcgccaataacctcaccagcaccatccaggtgtttacggactcggagtaccagctgccgtacgttctcggctctgcccaccagggctgcctgcctccgttcccggcggacgtgttcatgattccccagtacggctacctaacactcaacaacggtagtcaggccgtgggacgctcctccttctactgcctggaatactttccttcgcagatgctgagaaccggcaacaacttccagtttacttacaccttcgaggacgtgcctttccacagcagctacgcccacagccagagcttggaccggctgatgaatcctctgattgaccagtacctgtactacttgtctcggactcaaacaacaggaggcacggcaaatacgcagactctgggcttcagccaaggtgggcctaatacaatggccaatcaggcaaagaactggctgccaggaccctgttaccgccaacaacgcgtctcaacgacaaccgggcaaaacaacaatagcaactttgcctggactgctgggaccaaataccatctgaatggaagaaattcattggctaatcctggcatcgctatggcaacacacaaagacgacgaggagcgtttttttcccagtaacgggatcctgatttttggcaaacaaaatgctgccagagacaatgcggattacagcgatgtcatgctcaccagcgaggaagaaatcaaaaccactaaccctgtggctacagaggaatacggtatcgtggcagataacttgcagcagcaaaacacggctcctcaaattggaactgtcaacagccagggggccttacccggtatggtctggcagaaccgggacgtgtacctgcagggtcccatctgggccaagattcctcacacggacggcaacttccacccgtctccgctgatgggcggctttggcctgaaacatcctccgcctcagatcctgatcaagaacacgcctgtacctgcggatcctccgaccaccttcaaccagtcaaagctgaactctttcatcacgcaatacagcaccggacaggtcagcgtggaaattgaatgggagctgcagaaggaaaacagcaagcgctggaaccccgagatccagtacacctccaactactacaaatctacaagtgtggactttgctgttaatacagaaggcgtgtactctgaaccccgccccattggcacccgttacctcacccgtaatctg

SEQ ID NO: 23 - DNA, 165 bp, adeno-associated virus 2
ggaggggtggagtcgtgacgtgaattacgtcatagggttagggaggtcctgtattagaggtcacgtgagtgttttgcgacattttgcgacaccatgtggtctcgctgggggggggggcccgagtgagcacgcagggtctccattttgaagcgggaggtttgaacg

SEQ ID NO: 24 - DNA, 1866 bp, Artificial Sequence
  Nucleic acid sequence containing Rep region of serotype 2 AAV, synthetic sequence
acgccggggttttacgagattgtgattaaggtccccagcgaccttgacgagcatctgcccggcatttctgacagctttgtgaactgggtggccgagaaggaatgggagttgccgccagattctgacatggatctgaatctgattgagcaggcacccctgaccgtggccgagaagctgcagcgcgactttctgacggaatggcgccgtgtgagtaaggccccggaggcccttttctttgtgcaatttgagaagggagagagctacttccacatgcacgtgctcgtggaaaccaccggggtgaaatccatggttttgggacgtttcctgagtcagattcgcgaaaaactgattcagagaatttaccgcgggatcgagccgactttgccaaactggttcgcggtcacaaagaccagaaatggcgccggaggcgggaacaaggtggtggatgagtgctacatccccaattacttgctccccaaaacccagcctgagctccagtgggcgtggactaatatggaacagtatttaagcgcctgtttgaatctcacggagcgtaaacggttggtggcgcagcatctgacgcacgtgtcgcagacgcaggagcagaacaaagagaatcagaatcccaattctgatgcgccggtgatcagatcaaaaacttcagccaggtacatggagctggtcgggtggctcgtggacaaggggattacctcggagaagcagtggatccaggaggaccaggcctcatacatctccttcaatgcggcctccaactcgcggtcccaaatcaaggctgccttggacaatgcgggaaagattatgagcctgactaaaaccgcccccgactacctggtgggccagcagcccgtggaggacatttccagcaatcggatttataaaattttggaactaaacgggtacgatccccaatatgcggcttccgtctttctgggatgggccacgaaaaagttcggcaagaggaacaccatctggctgtttgggcctgcaactaccgggaagaccaacatcgcggaggccatagcccacactgtgcccttctacgggtgcgtaaactggaccaatgagaactttcccttcaacgactgtgtcgacaagatggtgatctggtgggaggaggggaagatgaccgccaaggtcgtggagtcggccaaagccattctcggaggaagcaaggtgcgcgtggaccagaaatgcaagtcctcggcccagatagacccgactcccgtgatcgtcacctccaacaccaacatgtgcgccgtgattgacgggaactcaacgaccttcgaacaccagcagccgttgcaagaccggatgttcaaatttgaactcacccgccgtctggatcatgactttgggaaggtcaccaagcaggaagtcaaagactttttccggtgggcaaaggatcacgtggttgaggtggagcatgaattctacgtcaaaaagggtggagccaagaaaagacccgcccccagtgacgcagatataagtgagcccaaacgggtgcgcgagtcagttgcgcagccatcgacgtcagacgcggaagcttcgatcaactacgcagacaggtaccaaaacaaatgttctcgtcacgtgggcatgaatctgatgctgtttccctgcagacaatgcgagagaatgaatcagaattcaaatatctgcttcactcacggacagaaagactgtttagagtgctttcccgtgtcagaatctcaacccgtttctgtcgtcaaaaaggcgtatcagaaactgtgctacattcatcatatcatgggaaaggtgccagacgcttgcactgcctgcgatctggtcaatgtggatttggatgactgcatctttgaacaataa

SEQ ID NO: 25 - DNA, 16 bp, Artificial Sequence
  Nucleic acid sequence of primer SI-1, synthetic sequence
gccagccatctgttgt

SEQ ID NO: 26 - DNA, 16 bp, Artificial Sequence
  Nucleic acid sequence of primer SI-2, synthetic sequence
ggagtggcaccttcca

SEQ ID NO: 27 - DNA, 21 bp, Artificial Sequence
  Nucleic acid sequence of probe SI-1, synthetic sequence
tcccccgtgccttccttgacc

SEQ ID NO: 28 - DNA, 21 bp, Artificial Sequence
  Nucleic acid sequence of primer SI-3, synthetic sequence
ggaacccctagtgatggagtt

SEQ ID NO: 29 - DNA, 16 bp, Artificial Sequence
  Nucleic acid sequence of primer SI-4, synthetic sequence
cggcctcagtgagcga

SEQ ID NO: 30 - DNA, 21 bp, Artificial Sequence
  Nucleic acid sequence of probe SI-2, synthetic sequence
cactccctctctgcgcgctcg

SEQ ID NO: 31 - protein, 11 aa, Artificial Sequence
  amino acid sequence of CDR1 in the light chain of anti-hTfR antibody 1
QSLVHSNGNTY

SEQ ID NO: 32 - protein, 16 aa, Artificial Sequence
  amino acid sequence of CDR1 in the light chain of anti-hTfR antibody 2
RSSQSLVHSNGNTYLH

SEQ ID NO: 33 - protein, 6 aa, Artificial Sequence
  amino acid sequence of CDR2 in the light chain of anti-hTfR antibody 1
KVSNRF

SEQ ID NO: 34 - protein, 7 aa, Artificial Sequence
  amino acid sequence of CDR2 in the light chain of anti-hTfR antibody 2
KVSNRFS

SEQ ID NO: 35 - protein, 9 aa, Artificial Sequence
  amino acid sequence of CDR3 in the light chain of anti-hTfR antibody 3
SQSTHVPWT

SEQ ID NO: 36 - protein, 5 aa, Artificial Sequence
  amino acid sequence of CDR1 in the heavy chain of anti-hTfR antibody 1
NYWLG

SEQ ID NO: 37 - protein, 8 aa, Artificial Sequence
  amino acid sequence of CDR1 in the heavy chain of anti-hTfR antibody 2
GYSFMNYW

SEQ ID NO: 38 - protein, 8 aa, Artificial Sequence
  amino acid sequence of CDR2 in the heavy chain of anti-hTfR antibody 1
IYPGGDYP

SEQ ID NO: 39 - protein, 17 aa, Artificial Sequence
  amino acid sequence of CDR2 in the heavy chain of anti-hTfR antibody 2
DIYPGGDYPTYSEKFKV

SEQ ID NO: 40 - protein, 9 aa, Artificial Sequence
  amino acid sequence of CDR3 in the heavy chain of anti-hTfR antibody 1
SGNYDEVAY

SEQ ID NO: 41 - protein, 11 aa, Artificial Sequence
  amino acid sequence of CDR3 in the heavy chain of anti-hTfR antibody 2
ARSGNYDEVAY

SEQ ID NO: 42 - protein, 766 aa, Artificial Sequence
  An example of amino acid sequence of a conjugate of human I2S and the Fab region of the heavy chain of an anti-hTfR antibody
EVQLVQSGAEVKKPGESLKISCKGSGYSFMNYWLGWVRQMPGKGLEWMGDIYPGGDYPTYSEKFKVQVTISADKSISTAYLQLSSLKASDTAMYYCARSGNYDEVAYWGQGTLVTVSSASTKGPSVFPLAPSSKSTSGGTAALGCLVKDYFPEPVTVSWNSGALTSGVHTFPAVLQSSGLYSLSSVVTVPSSSLGTQTYICNVNHKPSNTKVDKKVEPKSCDKTHTGGGGSGGGGSGGGGSSETQANSTTDALNVLLIIVDDLRPSLGCYGDKLVRSPNIDQLASHSLLFQNAFAQQAVCAPSRVSFLTGRRPDTTRLYDFNSYWRVHAGNFSTIPQYFKENGYVTMSVGKVFHPGISSNHTDDSPYSWSFPPYHPSSEKYENTKTCRGPDGELHANLLCPVDVLDVPEGTLPDKQSTEQAIQLLEKMKTSASPFFLAVGYHKPHIPFRYPKEFQKLYPLENITLAPDPEVPDGLPPVAYNPWMDIRQREDVQALNISVPYGPIPVDFQRKIRQSYFASVSYLDTQVGRLLSALDDLQLANSTIIAFTSDHGWALGEHGEWAKYSNFDVATHVPLIFYVPGRTASLPEAGEKLFPYLDPFDSASQLMEPGRQSMDLVELVSLFPTLAGLAGLQVPPRCPVPSFHVELCREGKNLLKHFRFRDLEEDPYLPGNPRELIAYSQYPRPSDIPQWNSDKPSLKDIKIMGYSIRTIDYRYTVWVGFNPDEFLANFSDIHAGELYFVDSDPLQDHNMYNDSQGGDLFQLLMP

SEQ ID NO: 43 - DNA, 589 bp, Artificial Sequence
  A preferable example of nucleic acid sequence of the first Long Terminal Repeat (first LTR) , synthetic sequence
tttgaaagaccccacccgtaggtggcaagctagcttaagtaacgccactttgcaaggcatggaaaaatacataactgagaatagaaaagttcagatcaaggtcaggaacaaagaaacagctgaataccaaacaggatatctgtggtaagcggttcctgccccggctcagggccaagaacagatgagacagctgagtgatgggccaaacaggatatctgtggtaagcagttcctgccccggctcggggccaagaacagatggtccccagatgcggtccagccctcagcagtttctagtgaatcatcagatgtttccagggtgccccaaggacctgaaaatgaccctgtaccttatttgaactaaccaatcagttcgcttctcgcttctgttcgcgcgcttccgctctccgagctcaataaaagagcccacaacccctcactcggcgcgccagtcttccgatagactgcgtcgcccgggtacccgtattcccaataaagcctcttgctgtttgcatccgaatcgtggtctcgctgttccttgggagggtctcctctgagtgattgactacccacgacgggggtctttcatt

SEQ ID NO: 44 - DNA, 594 bp, Artificial Sequence
  A preferable example of nucleic acid sequence of the second Long Terminal Repeat (second LTR) , synthetic sequence
aatgaaagaccccacctgtaggtttggcaagctagcttaagtaacgccattttgcaaggcatggaaaaatacataactgagaatagagaagttcagatcaaggtcaggaacagatggaacagctgaatatgggccaaacaggatatctgtggtaagcagttcctgccccggctcagggccaagaacagatggaacagctgaatatgggccaaacaggatatctgtggtaagcagttcctgccccggctcagggccaagaacagatggtccccagatgcggtccagccctcagcagtttctagagaaccatcagatgtttccagggtgccccaaggacctgaaatgaccctgtgccttatttgaactaaccaatcagttcgcttctcgcttctgttcgcgcgcttctgctccccgagctcaataaaagagcccacaacccctcactcggggcgccagtcctccgattgactgagtcgcccgggtacccgtgtatccaataaaccctcttgcagttgcatccgacttgtggtctcgctgttccttgggagggtctcctctgagtgattgactacccgtcagcgggggtctttcatt

SEQ ID NO: 45 - DNA, 52 bp, Sendai virus
accaaacaagagaagaaacttgtttggaatatataatgaagttagacaggat

SEQ ID NO: 46 - DNA, 54 bp, Sendai virus
acaaggagacaagaaaatttgaaagaataaatatctcttaaactcttgtctggt

SEQ ID NO: 47 - DNA, 4578 bp, Artificial Sequence
  Nucleic acid sequence of the DNA fragment synthesized for construction of pAAV-mMAP-Fab-hGLB1 vector, synthetic sequence
atcgatatcaagcttagatcattttgatggcagagttcagtttaccgggtcacattgtacctgggaagattcaaggatttatggaaaaagtcaacaacaggagtcagagcagccggaaaagcatggactctgtacttaggactgcgctttgagcaatggcacagcaagctataaccctgtttgcagtcagcacacaaactgtggttcaaagctccactttatctcttcttgtggaattcagatatcagatcagttttgctcaaatgggagacaaagagattaagctcttatgtaaaatttgctgttttacataactttaatgaatggacaaagtcttgtgcatgggggtgggggtggggttagaggggaacagctccagatggcaaacatacgcaagggatttagtcaaacaactttttggcaaagatggtatgattttgtaatggggtaggaaccaatgaaatgcgaggtaagtatggttaataatctacagttattggttaaagaagtatattagagcgagtctttctgcacacagatcaccttcctatcaaccccactagcctctggcaaaggtaccagtgtacagggagtcgctgcgttgccttcgccccgtgccccgctccgcgccgcctcgcgccgcccgccccggctctgactgaccgcgttactcccacaggtgagcgggcgggacggcccttctcctccgggctgtaattagcaagaggtaagggtttaagggatggttggttggtggggtattaatgtttaattacctggagcacctgcctgaaatcactttttttcaggttggacgcgtcgccaccatgggttggagcctcatcttgctcttccttgtcgctgttgctacgcgagtcggcagcgaggtgcaactagtgcagtctggagcagaggtgaaaaagcccggggagtctctgaagatttcctgtaagggttctggatacagctttatgaactactggctgggatgggtgcgccagatgcccgggaaaggcctggagtggatgggggacatctaccccggcggagactaccctacatacagcgagaagttcaaggtccaggtcaccatctcagccgacaagtccatcagcaccgcctacctgcagttgagcagcctgaaggcctcggacaccgccatgtattactgtgcgagatcaggcaattacgacgaagtggcctactggggccaaggaaccctggtcaccgtctcctcagctagcaccaagggcccatcggtcttccccctggcaccctcctccaagagcacctctgggggcacagcggccctgggctgcctggtcaaggactacttccccgaaccggtgacggtgtcgtggaactcaggcgccctgaccagcggcgtgcacaccttcccggctgtcctacagtcctcaggactctactccctcagcagcgtggtgaccgtgccctccagcagcttgggcacccagacctacatctgcaacgtgaatcacaagcccagcaacaccaaggtggacaagaaagttgagccgaagagctgtgataagacgcatacgggtggcggagggtctggaggtggcggatcaggcggaggtggatctcagaggatgttcgaaattgattactcccgggatagcttcctcaaagacggccagccttttaggtacatctccggctccattcactattcccgggtgcctcgtttttactggaaagaccggctgctgaagatgaagatggccggactgaacgctatccagacctacgtcccttggaactttcatgagccttggcccggccagtaccaatttagcgaggaccacgacgtcgagtactttttacggctggcccacgaactcggactcctcgtgattctgaggcccggcccctacatttgcgccgagtgggagatgggaggtttacccgcttggctgctggagaaggagtccatcttattacggagcagcgatcccgattatttagccgccgtggacaaatggctgggagttttactccccaagatgaaacctttactgtaccagaatggcggccccgttatcaccgtccaagttgagaatgagtatggctcctatttcgcttgcgacttcgactatttacggtttttacagaagaggtttcgtcaccacctcggagacgatgtcgtcctcttcaccaccgatggagcccataagacctttttaaagtgtggcgccctccaaggtttatataccaccgtggatttcggcactggtagcaacatcacagatgcctttctctcccagcggaagtgcgaacctaagggccctttaatcaattccgagttctacaccggctggctcgaccactggggccagcctcactccaccatcaagacagaagccgtggccagctctttatacgacatcctcgctcggggcgcctccgtcaatttatacatgtttatcggcggcaccaacttcgcctattggaacggcgctaactccccctacgccgctcagcccacaagctatgactatgatgcccctctgtccgaagccggagatttaaccgagaagtacttcgccctccggaacatcattcagaagttcgagaaggtgcccgagggacccatccctcccagcacccccaagttcgcttacggaaaagtcaccctcgaaaaactgaagaccgtgggcgccgctttagatattctgtgccccagcggccctattaagtctttataccccctcacctttattcaagttaagcagcattacggctttgttttataccggaccactttaccccaagattgtagcaaccccgctcctctgagcagccctttaaacggcgtccatgatcgggcttatgtggctgtcgacggcattccccaaggtgtgctcgaacggaacaacgtgatcactttaaatatcaccggcaaagctggcgctacactggatctgctggtcgaaaacatgggccgggtgaactacggcgcctacattaacgatttcaagggtttagtgtccaatttaacactcagctccaacattctcaccgactggaccatcttccctttagacaccgaggatgctgtgaggagccatttaggcggatggggccatcgggacagcggacatcacgacgaggcttgggctcacaatagctccaactacacactgcccgctttctacatgggcaacttcagcatccctagcggaattcccgatctgcctcaagataccttcatccaattccccggctggaccaagggccaagtttggatcaacggctttaatttaggccggtactggcccgctcgtggacctcagctgacactgttcgtgcctcaacacattttaatgacctccgctcctaacacaatcaccgtgctggagctggagtgggctccttgtagctccgacgatcccgagctgtgcgccgtcaccttcgtcgatcgtcccgtcatcggctcctccgtgacatacgaccaccccagcaagcccgttgagaagcggctgatgcctcctcctcctcagaagaacaaggactcttggctggaccacgtgggaagcggagctactaacttcagcctgctgaagcaggctggagacgtggaggagaaccctggacctatgggctggagctggattctgctgttcctcctgagcgtgacagcaggagtgcacagcgacatcgtgatgacccagactcccctgagcctgagcgtgacacctggccagcctgccagcatcagctgcagaagctctcagagcctggtgcacagcaacggcaacacctacctgcactggtatctgcagaagcccggccagagccctcagctgctgatctacaaggtgtccaacagattcagcggcgtgcccgacagattctccggcagcggctctggcaccgacttcaccctgaagatttccagagtggaagccgaggacgtgggcgtgtactactgcagccagagcacccacgtgccctggacattcggccagggcaccaaggtggaaatcaagagaaccgtggccgctcccagcgtgttcatcttcccacctagcgacgagcagctgaagtccggcacagcctctgtcgtgtgcctgctgaacaacttctacccccgcgaggccaaggtgcagtggaaggtggacaacgccctgcagagcggcaacagccaggaaagcgtgaccgagcaggactccaaggacagcacctacagcctgagcagcaccctgaccctgagcaaggccgactacgagaagcacaaggtgtacgcctgcgaagtgacccaccagggcctgtctagccccgtgaccaagagcttcaacagaggcgagtgctaataaatttaaatgcggccgcatttaaatctgtgccttctagttgccagccatctgttgtttgcccctcccccgtgccttccttgaccctggaaggtgccactcccactgtcctttcctaataaaatgaggaaattgcatcgcattgtctgagtaggtgtcattctattctggggggtggggtggggcaggacagcaagggggaggattgggaagacaatagcaggcatgctggggaagatct

SEQ ID NO: 48 - protein, 890 aa, Artificial Sequence
  An example of amino acid sequence of a conjugate of human  À-galactosidase and the Fab region of the heavy chain of an anti-hTfR antibody
EVQLVQSGAEVKKPGESLKISCKGSGYSFMNYWLGWVRQMPGKGLEWMGDIYPGGDYPTYSEKFKVQVTISADKSISTAYLQLSSLKASDTAMYYCARSGNYDEVAYWGQGTLVTVSSASTKGPSVFPLAPSSKSTSGGTAALGCLVKDYFPEPVTVSWNSGALTSGVHTFPAVLQSSGLYSLSSVVTVPSSSLGTQTYICNVNHKPSNTKVDKKVEPKSCDKTHTGGGGSGGGGSGGGGSQRMFEIDYSRDSFLKDGQPFRYISGSIHYSRVPRFYWKDRLLKMKMAGLNAIQTYVPWNFHEPWPGQYQFSEDHDVEYFLRLAHELGLLVILRPGPYICAEWEMGGLPAWLLEKESILLRSSDPDYLAAVDKWLGVLLPKMKPLLYQNGGPVITVQVENEYGSYFACDFDYLRFLQKRFRHHLGDDVVLFTTDGAHKTFLKCGALQGLYTTVDFGTGSNITDAFLSQRKCEPKGPLINSEFYTGWLDHWGQPHSTIKTEAVASSLYDILARGASVNLYMFIGGTNFAYWNGANSPYAAQPTSYDYDAPLSEAGDLTEKYFALRNIIQKFEKVPEGPIPPSTPKFAYGKVTLEKLKTVGAALDILCPSGPIKSLYPLTFIQVKQHYGFVLYRTTLPQDCSNPAPLSSPLNGVHDRAYVAVDGIPQGVLERNNVITLNITGKAGATLDLLVENMGRVNYGAYINDFKGLVSNLTLSSNILTDWTIFPLDTEDAVRSHLGGWGHRDSGHHDEAWAHNSSNYTLPAFYMGNFSIPSGIPDLPQDTFIQFPGWTKGQVWINGFNLGRYWPARGPQLTLFVPQHILMTSAPNTITVLELEWAPCSSDDPELCAVTFVDRPVIGSSVTYDHPSKPVEKRLMPPPPQKNKDSWLDHV

SEQ ID NO: 49 - DNA, 66 bp, Porcine teschovirus-1
ggaagcggagctactaacttcagcctgctgaagcaggctggagacgtggaggagaaccctggacct

SEQ ID NO: 50 - protein, 649 aa, Homo sapiens
QRMFEIDYSRDSFLKDGQPFRYISGSIHYSRVPRFYWKDRLLKMKMAGLNAIQTYVPWNFHEPWPGQYQFSEDHDVEYFLRLAHELGLLVILRPGPYICAEWEMGGLPAWLLEKESILLRSSDPDYLAAVDKWLGVLLPKMKPLLYQNGGPVITVQVENEYGSYFACDFDYLRFLQKRFRHHLGDDVVLFTTDGAHKTFLKCGALQGLYTTVDFGTGSNITDAFLSQRKCEPKGPLINSEFYTGWLDHWGQPHSTIKTEAVASSLYDILARGASVNLYMFIGGTNFAYWNGANSPYAAQPTSYDYDAPLSEAGDLTEKYFALRNIIQKFEKVPEGPIPPSTPKFAYGKVTLEKLKTVGAALDILCPSGPIKSLYPLTFIQVKQHYGFVLYRTTLPQDCSNPAPLSSPLNGVHDRAYVAVDGIPQGVLERNNVITLNITGKAGATLDLLVENMGRVNYGAYINDFKGLVSNLTLSSNILTDWTIFPLDTEDAVRSHLGGWGHRDSGHHDEAWAHNSSNYTLPAFYMGNFSIPSGIPDLPQDTFIQFPGWTKGQVWINGFNLGRYWPARGPQLTLFVPQHILMTSAPNTITVLELEWAPCSSDDPELCAVTFVDRPVIGSSVTYDHPSKPVEKRLMPPPPQKNKDSWLDHV